European Patent Specification EP 3 377 603 B1, published February 14, 2024. Title: PREPARATION OF A STABLE BEVERAGE. Applicant: DSM IP Assets B.V. The sequence listing filed with the application follows.

SEQUENCE LISTING (3 sequences)

SEQ ID NO: 1 - DNA, 1580 bp, Artificial Sequence
  source 1..1580: /organism="Artificial Sequence" /note="Codon optimized nucleic acid encoding proline-specific endoprotease from Rasamsonia emersonii PEP-R.e.for expression in A. niger" /mol_type="unassigned DNA"
atgccctccctctcctccctcgttgccttgactgcttctcttgtctctctggctgctgccgctgctcctcgtctccctcttcctcctcgccctcccttgcctccccgtgaccccttgcacggacctaccaacgcctccgccactttccagcagctcatcgaccacaaccaccccgagcttggcaccttctcccagcgctactggtggaatgatgagttctggaagggtcccggctctcccgttgtccttttcacccccggtgaagaagatgccagcggttacgtgggctacctgaagaacaccaccatcaccggtctgatcgctcagaccatcggtggtgccgtcatcgtcctcgaacaccgctactggggccagtcctccccctacgactctctgaccaccaagaacctgcagtacctgaccctcaagcagtccattgccgacctcacctacttcgccaagaccgtcaagctccccttcgaccgcaacggcagctccaacgccgacaaggctccctgggttctcagcggtggaagctactctggtgctctctccgcctggactgccagcacctcccccggtactttctgggcctaccacgccagctctgctcctgttgaggccatctacgattactggcagtacttcgctcccgtgcaggatggattgcctgccaactgctcgaaggacctctcccgtgtcgtcgactacatcgactccgttctccagtccggcaacgccactgccaagcaacagctcaaggaccttttcggtctgggtgctctggagcacgacgatgacttcgcctccgctcttgagaacggcccttggctctggcagtcgaactcgttctacgacccctaccctcctgtctacgagttctgcgactacgttgagaacgcctacgccagccctcccgttgctgctggtcccgatggtgttggtctggagaaggctctgtctggctacgccacctggtggaacaaggtcttcttccccggctactgcgctacctacggctactggtcctccaacgactccattgcctgcttcgacacctacaaccagtcgtcgcccatgttcaccgacctttccgtctccaacactatcaaccgccagtggaactggttcctctgcaacgagcccttcttctactggcaggatggtgctcccaagaacgtccccagcattgtctctcgtctggtcactgctgagtactggcagcgccagtgccccttgttcttccctgaagaggatggctacacctacggaagcgccaagggcaagactgctgccgatgtcaacgcctggaccaagggctggttcttgactaacaccacccgtctgatctggaccaacggcgagcttgacccctggcgctctgctggtgtcagcagcaagttccgtcccggtggtcccctccagtccactccccaggctcctctgcagctcattcccgagggtgtccactgctacgatctgatcctcaagaacgccgaggccaacgccggtgtgcagcgtgttgtcaccaacgaggttgctcagatcaaggcctgggtgaacgaatactaccgtaagta

SEQ ID NO: 2 - protein, 526 aa, Artificial Sequence
  Rasamsonia emersonii
MPSLSSLVALTASLVSLAAAAAPRLPLPPRPPLPPRDPLHGPTNASATFQQLIDHNHPELGTFSQRYWWNDEFWKGPGSPVVLFTPGEEDASGYVGYLKNTTITGLIAQTIGGAVIVLEHRYWGQSSPYDSLTTKNLQYLTLKQSIADLTYFAKTVKLPFDRNGSSNADKAPWVLSGGSYSGALSAWTASTSPGTFWAYHASSAPVEAIYDYWQYFAPVQDGLPANCSKDLSRVVDYIDSVLQSGNATAKQQLKDLFGLGALEHDDDFASALENGPWLWQSNSFYDPYPPVYEFCDYVENAYASPPVAAGPDGVGLEKALSGYATWWNKVFFPGYCATYGYWSSNDSIACFDTYNQSSPMFTDLSVSNTINRQWNWFLCNEPFFYWQDGAPKNVPSIVSRLVTAEYWQRQCPLFFPEEDGYTYGSAKGKTAADVNAWTKGWFLTNTTRLIWTNGELDPWRSAGVSSKFRPGGPLQSTPQAPLQLIPEGVHCYDLILKNAEANAGVQRVVTNEVAQIKAWVNEYYRK

SEQ ID NO: 3 - DNA, 13 bp, Artificial Sequence
  source 1..13: /organism="Artificial Sequence" /note="Translation initiation sequence of glaA promotor" /mol_type="unassigned DNA"
caccgtcaaaatg